European Patent Specification EP 4 090 763 B1, published December 4, 2024. Title: METHODS AND COMPOSITIONS FOR QUANTITATION OF PROTEINS AND RNA. Applicant: Becton, Dickinson and Company Prosen, Dennis Lazaruk, Katherine. The sequence listing filed with the application follows.

SEQUENCE LISTING (11 sequences)

SEQ ID NO: 1 - DNA, 95 bp, Artificial Sequence
  Synthetic Oligonucleotide
  5'AmMC6 (1)..(1): 5' Amino Modifier C6
gttgtcaagatgctaccgttcagagtacgtggagttggtggcccgaccccgagcgctacgagccccccggaaaaaaaaaaaaaaaaaaaaaaaaa

SEQ ID NO: 2 - DNA, 200 bp, Artificial Sequence
  Synthetic Oligonucleotide
  5AmMC6 (1)..(1): 5' Amino Modifier C6
gttgtcaagatgctaccgttcagagctactgtccgaagttaccgtgtatctaccacgggtggtttttcgaatccggaaaagatagtaataagtgttttagttggaataagtcgcaacttttggagacggttacctctcaatttttctgatccgtaggccccccgatctcggcctcaaaaaaaaaaaaaaaaaaaaaaaaa

SEQ ID NO: 3 - DNA, 25 bp, Artificial Sequence
  Synthetic Oligonucleotide
gttgtcaagatgctaccgttcagag

SEQ ID NO: 4 - DNA, 20 bp, Artificial Sequence
  Synthetic Oligonucleotide
acacgacgctcttccgatct

SEQ ID NO: 5 - DNA, 95 bp, Artificial Sequence
  Synthetic Oligonucleotide
gttgtcaagatgctaccgttcagagccccatgtctagtacctattggtcccctatcctcagattcgtttaaaaaaaaaaaaaaaaaaaaaaaaaa

SEQ ID NO: 6 - DNA, 26 bp, Artificial Sequence
  Synthetic Oligonucleotide
tttttttttttttttttttttttttt

SEQ ID NO: 7 - DNA, 95 bp, Artificial Sequence
  Synthetic Oligonucleotide
  5AmMC12 (1)..(1): 5' Amino Modifier C12
gttgtcaagatgctaccgttcagagattcaagggcagccgcgtcacgattggatacgactgttggaccggaaaaaaaaaaaaaaaaaaaaaaaaa

SEQ ID NO: 8 - DNA, 102 bp, Artificial Sequence
  Synthetic Oligonucleotide
  5'AmMC12 (1)..(1): 5' Amino Modifier C12
  misc_feature (24)..(25): n is a, c, g, or t
  misc_feature (27)..(30): n is a, c, g, or t
  misc_feature (32)..(33): n is a, c, g, or t
  misc_feature (35)..(75): n is a, c, g, or t
cagacgtgtgctcttccgatctvnnvnnnnvnnvnnnnnnnnnnnnnnnnnnnnnnnnnnnnnnnnnnnnnnnnnbbaaaaaaaaaaaaaaaaaaaaaaaaa

SEQ ID NO: 9 - DNA, 100 bp, Artificial Sequence
  Bead Oligonucleotide
  misc_feature (23)..(31): n is a, c, g, or t
  misc_feature (44)..(52): n is a, c, g, or t
  misc_feature (66)..(82): n is a, c, g, or t
ctacacgacgctcttccgatctnnnnnnnnnactggcctgcgannnnnnnnnggtagcggtgacannnnnnnnnnnnnnnnntttttttttttttttttt

SEQ ID NO: 10 - DNA, 95 bp, Artificial Sequence
  AbSeq Oligonucleotide
  misc_feature (24)..(25): n is a, c, g, or t
  misc_feature (27)..(30): n is a, c, g, or t
  misc_feature (32)..(33): n is a, c, g, or t
cagacgtgtgctcttccgatctvnnvnnnnvnnvcggcatgaattaggcgagacttagtatacgagctggaaaaaaaaaaaaaaaaaaaaaaaaa

SEQ ID NO: 11 - DNA, 22 bp, Artificial Sequence
  Abseq PCR1 primer (pR2)
cagacgtgtgctcttccgatct